European Patent Specification EP 3 740 504 B1, published July 19, 2023. Title: CD70 COMBINATION THERAPY. Applicant: ARGENX BVBA. The sequence listing filed with the application follows.

SEQUENCE LISTING (136 sequences)

SEQ ID NO: 1 - protein, 5 aa, Artificial
  Synthetic peptide
VYYMN

SEQ ID NO: 2 - protein, 17 aa, Artificial
  Synthetic peptide
DINNEGGTTYYADSVKG

SEQ ID NO: 3 - protein, 13 aa, Artificial
  Synthetic peptide
DAGYSNHVPIFDS

SEQ ID NO: 4 - protein, 122 aa, Artificial
  Synthetic peptide
EVQLVESGGGLVQPGGSLRLSCAASGFTFSVYYMNWVRQAPGKGLEWVSDINNEGGTTYYADSVKGRFTISRDNSKNSLYLQMNSLRAEDTAVYYCARDAGYSNHVPIFDSWGQGTLVTVSS

SEQ ID NO: 5 - protein, 14 aa, Artificial
  Synthetic peptide
GLKSGSVTSDNFPT

SEQ ID NO: 6 - protein, 7 aa, Artificial
  Synthetic peptide
NTNTRHS

SEQ ID NO: 7 - protein, 10 aa, Artificial
  Synthetic peptide
ALFISNPSVE

SEQ ID NO: 8 - protein, 111 aa, Artificial
  Synthetic peptide
QAVVTQEPSLTVSPGGTVTLTCGLKSGSVTSDNFPTWYQQTPGQAPRLLIYNTNTRHSGVPDRFSGSILGNKAALTITGAQADDEAEYFCALFISNPSVEFGGGTQLTVLG

SEQ ID NO: 9 - protein, 123 aa, Artificial
  Synthetic peptide
EVQLVESGGGLVQPGGSLRLSCAASGFTFSSYAMSWVRQAPGKGPEWVSHINSGGGNTKYADSVKGRFTISRDNAKNTLYLQMNTLKPEDTAVYYCAKDVSGGYYGTYALDAWGQGTQVVVSS

SEQ ID NO: 10 - protein, 106 aa, Artificial
  Synthetic peptide
SYELTQSPSVSVALKQTAKITCGGDNIGSKSAQWYQQKPGQAPVLVIYADSRRPSGIPERFSGSNSGNTATLTISGAQAEDEADYYCQVWDSSAAVFGGGTHLTVL

SEQ ID NO: 11 - protein, 121 aa, Artificial
  Synthetic peptide
EVQVQESGGGLVQPGGSLRLSCAASGFTFSSYAMSWVRQAPGKGLEWVSDINSGGGSTVYTDSVKGRFTISRDNAKNTLYLQMNSLKPDDTAVYYCATGGSYYSYRLFDYWGQGTQVTVSS

SEQ ID NO: 12 - protein, 114 aa, Artificial
  Synthetic peptide
DIQMTQSPSSVIVSAGEKVTINCKSSQSVLDSSNQKNYLAWYQQRLGQSPRLLIYWASTRESGVPDRFSGSGSTTDFTLTISSFQPEDAAVYYCQQGYSVPVTFGQGTKVELKR

SEQ ID NO: 13 - protein, 124 aa, Artificial
  Synthetic peptide
QVQLVESGGGLVQPGGSLRLSCAASGFTFSNYWMYWVRQAPGKGLEWVSTINTNGAITLYADNVKDRFTVSRDNAKNTLYLQMNSLKSEDTAVYYCAKVKLSGYPHPYYAMDYWGKGTLVTVSS

SEQ ID NO: 14 - protein, 115 aa, Artificial
  Synthetic peptide
NFMLTQPPSLSGSLGQSARLTCTLGSGNSIGAHTISWYQQKAGSPPRYLLNYYSDSSNHQASGVPSRFSGSKDDSTNAGLLLISGLQPEDEADYYCAAGDGSGTVFGGGTKLTVL

SEQ ID NO: 15 - protein, 122 aa, Artificial
  Synthetic peptide
QVQLVESGPGLVKPSQTLSLTCTVSGGSITTSDDAWSWIRQPAGKGLEWMGVIAYDGSTRYSPSLQSRTSISRDTSKNQFSLQLSSVTPEDTAVYYCARTKGVGGTWALDAWGQGTLVTVSS

SEQ ID NO: 16 - protein, 114 aa, Artificial
  Synthetic peptide
EIVLTQSPSSVTASVGEKVTINCKSSQSVLSSSNQKNYLSWYQQRLGQSPRLLITWASTRESGVPDRFSGSGSTTDFTLTISSFQPEDAAVYYCQQGYGAPLTFGQGTKVELKR

SEQ ID NO: 17 - protein, 122 aa, Artificial
  Synthetic peptide
QVQLVESGGGLVQPGGSLRLSCAASGFAFSSYDMSWVRQAPGKGLEWVSTINSGGGSTNYADSMKGRFTISRDNAKNTVYLQMNSLKPEDTAVYYCAARSPYYTRVPLYDYWGQGTQVTVSS

SEQ ID NO: 18 - protein, 110 aa, Artificial
  Synthetic peptide
QAVVTQEPSLSVSLGGTVTLTCGLRSGSVTTSNYPGWFKQTPGQAPRTLIFGASSRHSGVPSRYSGSISGNKAALTITGAEPEDEADYYCALNKGTYTDVFGGGTKLTVL

SEQ ID NO: 19 - protein, 125 aa, Artificial
  Synthetic peptide
EVQLQESGPGLVKPSQTLSLTCTVSGASVTTRYNYWSWIRQPPGKGLEWMGAITYSGSTYYSPSLKSRTSISRDTSKNQFTLQLSSVTPEDTAVYYCATEGSSSTGVSRYSFGSWGQGTQVTVSS

SEQ ID NO: 20 - protein, 111 aa, Artificial
  Synthetic peptide
ATMLTQSPGSLSVVPGESASISCKASQSLTHTDGTTALYWLQQKPGQRPQLLIYEVSVRASGVPDRFTGSGSGSDFTLKINGVKAEDAGVYYCAQVAYYPTFGQGTKVELK

SEQ ID NO: 21 - protein, 118 aa, Artificial
  Synthetic peptide
QVQLQESGPGLVKPSQTLSLTCTVSGGSITTNRYLWTWIRQTPGKGLEWVGAIAYSGRTYYSPSLKSRTSISRDTSKNQFTLQLSSVTPEDTGVYYCAHFTGWGGYYWGQGTQVTVSS

SEQ ID NO: 22 - protein, 110 aa, Artificial
  Synthetic peptide
QSALTQPPSVSGTLGKTVTISCAGTSSDIGGYNSVSWYQQLPGTAPKLLIYEVNKRASGIPDRFSGSKSGNTASLSISGLQSEDEADYYCASYRSANNVVFGGGTKLTVL

SEQ ID NO: 23 - protein, 122 aa, Artificial
  Synthetic peptide
QVQLVESGGGLVQPGGSLRLSCAASGFAFSSYDMSWVRQAPGKGPEWVSTINSGGGSTSYADSVKGRFTISRDNAKNTVYLQMNSLKPEDTAVYYCAARSLYYTRVPMYDYWGQGTQVTVSK

SEQ ID NO: 24 - protein, 110 aa, Artificial
  Synthetic peptide
QAVVTQEPSLSVSPGGTVTLTCGLSSGSVTTNNYPGWFQQTPGQAPRTLIYSTSSRHSGVPSRFSGSISGNKAALTITGAQPEDEADYYCALDIGSYTAVFGGGTHLTVL

SEQ ID NO: 25 - protein, 125 aa, Artificial
  Synthetic peptide
EVQLVQPGAELRNPGASVKVSCKASGYTFTMYYIDWVRQAPGQGLEWMGRIDPEDGGTKYAQKFQGRVTFTADTSTSTAYVELSSLRSEDTAVYYCARIPNGGSYYYTPYDYDYWGQGTQVTVSS

SEQ ID NO: 26 - protein, 110 aa, Artificial
  Synthetic peptide
QAVVTQEPSLSVSPGGTVTLTCGLTSGSVTSSNYPGWYRQTPGQAPRPLIYNTNSRHPGVPSRYSGSISENKATLTITGAEPEDEADYYCALHKGSYTAVFGGGTHLTVL

SEQ ID NO: 27 - protein, 121 aa, Artificial
  Synthetic peptide
QVQLQESGGGLVQPGGSLTLSCAASGFFFSSYAMSWVRQAPGKGLEWVSSISAGGGTSYYADSVKGRFTISRDSAKNTLVLQMNSLKPEDTAVYYCAKKRQNFWSEGYDSWGQGTQVTVSS

SEQ ID NO: 28 - protein, 110 aa, Artificial
  Synthetic peptide
HSAVTQPPSVSGSPGKAVTISCVGSSSDVGYGDYVSWYQQLPGMAPKLLIYDVEKRASGIPDRFSGSKSGNTASLTISGLQSEDEADYYCASYRSDSNFVFGGGTHLAVL

SEQ ID NO: 29 - protein, 120 aa, Artificial
  Synthetic peptide
QLQLVESGGGLVQPGGSLRLSCAASGFTFGSYDMSWVRQAPGKGPEWVSRITSGGGSTYADSVKGRFTISRDNAKNTLSLQMNSLKSEDTAVYYCAAGQYSDGYYPYDYWGQGTQVTVSS

SEQ ID NO: 30 - protein, 107 aa, Artificial
  Synthetic peptide
DIVMTQSPSSLSASLGDRVTITCQASQSISSYLAWYQQKPGQGPKLLIYGASRLEPGVPSRFSGSGSGTSFTLTISGVEAEDLATYYCLQDYSWPYSFGSGTRLEIK

SEQ ID NO: 31 - protein, 114 aa, Artificial
  Synthetic peptide
ELQVVESGGGLVQPGGSLRLSCAASGFTFGSYDMSWHRQAPRKGPEWVSTISAGGGRTYYADSVKGRFTISRDNAKNTLYLQMNSLKPEDTAVYFCTKIVLDSWGQGTQVTVSS

SEQ ID NO: 32 - protein, 111 aa, Artificial
  Synthetic peptide
DVVLTQTPGSLSVVPGESASISCKASQSLIHIDGKTYLYWLLQKPGRRPELLIYQVSNHESGVPDRFTGSGSGTDFTLKISGVKAEDAGVYYCAQATYYPSFGSGTRLEIK

SEQ ID NO: 33 - protein, 117 aa, Artificial
  Synthetic peptide
EVQLVESGGGLVQPGGSLRLSCAASGFTFDDYTMSWVRQVPGKGLEWISGISGNGGRTDYVEPIEGRFTISRDNAKNTLYLQMNSLKSEDTAVYYCAKTSPQSLDYWGQGTQVTVSS

SEQ ID NO: 34 - protein, 113 aa, Artificial
  Synthetic peptide
DIVMTQSPSSVTASVGEKVTINCKSSQSVVSGSNQKSYLNWYQQRPGQPPRLLIYYASTQESGIPDRFSGSGSTTDFTLTISSVQPEDAAVYYCQQAYSAPYNFGSGTRLEIK

SEQ ID NO: 35 - protein, 114 aa, Artificial
  Synthetic peptide
EVQLVESGGGLVQPGGSLRLSCAASGFTFGSYDMSWVRQAPGKGPEWVSTISAGGGRTYYADSVKDRFTISRDNAKNTLYLQMNSLKPEDTAVYYCAKVVIDYWGQGTQVTVSS

SEQ ID NO: 36 - protein, 111 aa, Artificial
  Synthetic peptide
DVVLTQTPGSLSVVPGESASISCKASQSLVHTDGKTYVYWLLQKPGQRPHLLIYQVSNHESGVPDRFTGSGSGTDFTLKISGVKAEDAGVYYCAQATYYPSFGSGTRLEIK

SEQ ID NO: 37 - protein, 125 aa, Artificial
  Synthetic peptide
EVQLVESGGGLVQPGGSLRLSCAASGFTFSSYSMSWVRQAPGKGPEWVSGINTSGGTTSYAASVKGRFTVSRDNAKNTLSLQMNSLEPEDTAVYYCVKHIRWSGSNYYYYGMDYWGKGTLVTVSS

SEQ ID NO: 38 - protein, 110 aa, Artificial
  Synthetic peptide
QAVLTQPPSVSGSPGQRFTISCTGSNRNIGNNYVNWYQQLPGTAPKLLIYSDNLRTSGVPARFSASKSGTTSSLTISGLQAEDEAVYYCSSWDDSLSGAVFGGGTHLTVL

SEQ ID NO: 39 - protein, 5 aa, Artificial
  Synthetic peptide
SYAMS

SEQ ID NO: 40 - protein, 17 aa, Artificial
  Synthetic peptide
HINSGGGNTKYADSVKG

SEQ ID NO: 41 - protein, 14 aa, Artificial
  Synthetic peptide
DVSGGYYGTYALDA

SEQ ID NO: 42 - protein, 17 aa, Artificial
  Synthetic peptide
DINSGGGSTVYTDSVKG

SEQ ID NO: 43 - protein, 12 aa, Artificial
  Synthetic peptide
GGSYYSYRLFDY

SEQ ID NO: 44 - protein, 5 aa, Artificial
  Synthetic peptide
NYWMY

SEQ ID NO: 45 - protein, 17 aa, Artificial
  Synthetic peptide
TINTNGAITLYADNVKD

SEQ ID NO: 46 - protein, 15 aa, Artificial
  Synthetic peptide
VKLSGYPHPYYAMDY

SEQ ID NO: 47 - protein, 7 aa, Artificial
  Synthetic peptide
TSDDAWS

SEQ ID NO: 48 - protein, 16 aa, Artificial
  Synthetic peptide
VIAYDGSTRYSPSLQS

SEQ ID NO: 49 - protein, 12 aa, Artificial
  Synthetic peptide
TKGVGGTWALDA

SEQ ID NO: 50 - protein, 5 aa, Artificial
  Synthetic peptide
SYDMS

SEQ ID NO: 51 - protein, 17 aa, Artificial
  Synthetic peptide
TINSGGGSTNYADSMKG

SEQ ID NO: 52 - protein, 13 aa, Artificial
  Synthetic peptide
RSPYYTRVPLYDY

SEQ ID NO: 53 - protein, 7 aa, Artificial
  Synthetic peptide
TRYNYWS

SEQ ID NO: 54 - protein, 16 aa, Artificial
  Synthetic peptide
AITYSGSTYYSPSLKS

SEQ ID NO: 55 - protein, 15 aa, Artificial
  Synthetic peptide
EGSSSTGVSRYSFGS

SEQ ID NO: 56 - protein, 7 aa, Artificial
  Synthetic peptide
TNRYLWT

SEQ ID NO: 57 - protein, 16 aa, Artificial
  Synthetic peptide
AIAYSGRTYYSPSLKS

SEQ ID NO: 58 - protein, 8 aa, Artificial
  Synthetic peptide
FTGWGGYY

SEQ ID NO: 59 - protein, 17 aa, Artificial
  Synthetic peptide
TINSGGGSTSYADSVKG

SEQ ID NO: 60 - protein, 13 aa, Artificial
  Synthetic peptide
RSLYYTRVPMYDY

SEQ ID NO: 61 - protein, 5 aa, Artificial
  Synthetic peptide
MYYID

SEQ ID NO: 62 - protein, 17 aa, Artificial
  Synthetic peptide
RIDPEDGGTKYAQKFQG

SEQ ID NO: 63 - protein, 16 aa, Artificial
  Synthetic peptide
IPNGGSYYYTPYDYDY

SEQ ID NO: 64 - protein, 17 aa, Artificial
  Synthetic peptide
SISAGGGTSYYADSVKG

SEQ ID NO: 65 - protein, 12 aa, Artificial
  Synthetic peptide
KRQNFWSEGYDS

SEQ ID NO: 66 - protein, 16 aa, Artificial
  Synthetic peptide
RITSGGGSTYADSVKG

SEQ ID NO: 67 - protein, 12 aa, Artificial
  Synthetic peptide
GQYSDGYYPYDY

SEQ ID NO: 68 - protein, 17 aa, Artificial
  Synthetic peptide
TISAGGGRTYYADSVKG

SEQ ID NO: 69 - protein, 5 aa, Artificial
  Synthetic peptide
IVLDS

SEQ ID NO: 70 - protein, 5 aa, Artificial
  Synthetic peptide
DYTMS

SEQ ID NO: 71 - protein, 17 aa, Artificial
  Synthetic peptide
GISGNGGRTDYVEPIEG

SEQ ID NO: 72 - protein, 8 aa, Artificial
  Synthetic peptide
TSPQSLDY

SEQ ID NO: 73 - protein, 17 aa, Artificial
  Synthetic peptide
TISAGGGRTYYADSVKD

SEQ ID NO: 74 - protein, 5 aa, Artificial
  Synthetic peptide
VVIDY

SEQ ID NO: 75 - protein, 5 aa, Artificial
  Synthetic peptide
SYSMS

SEQ ID NO: 76 - protein, 17 aa, Artificial
  Synthetic peptide
GINTSGGTTSYAASVKG

SEQ ID NO: 77 - protein, 16 aa, Artificial
  Synthetic peptide
HIRWSGSNYYYYGMDY

SEQ ID NO: 78 - protein, 11 aa, Artificial
  Synthetic peptide
GGDNIGSKSAQ

SEQ ID NO: 79 - protein, 7 aa, Artificial
  Synthetic peptide
ADSRRPS

SEQ ID NO: 80 - protein, 9 aa, Artificial
  Synthetic peptide
QVWDSSAAV

SEQ ID NO: 81 - protein, 17 aa, Artificial
  Synthetic peptide
KSSQSVLDSSNQKNYLA

SEQ ID NO: 82 - protein, 7 aa, Artificial
  Synthetic peptide
WASTRES

SEQ ID NO: 83 - protein, 9 aa, Artificial
  Synthetic peptide
QQGYSVPVT

SEQ ID NO: 84 - protein, 14 aa, Artificial
  Synthetic peptide
TLGSGNSIGAHTIS

SEQ ID NO: 85 - protein, 13 aa, Artificial
  Synthetic peptide
YYSDSSNHQASGV

SEQ ID NO: 86 - protein, 9 aa, Artificial
  Synthetic peptide
AAGDGSGTV

SEQ ID NO: 87 - protein, 17 aa, Artificial
  Synthetic peptide
KSSQSVLSSSNQKNYLS

SEQ ID NO: 88 - protein, 9 aa, Artificial
  Synthetic peptide
QQGYGAPLT

SEQ ID NO: 89 - protein, 14 aa, Artificial
  Synthetic peptide
GLRSGSVTTSNYPG

SEQ ID NO: 90 - protein, 7 aa, Artificial
  Synthetic peptide
GASSRHS

SEQ ID NO: 91 - protein, 10 aa, Artificial
  Synthetic peptide
ALNKGTYTDV

SEQ ID NO: 92 - protein, 16 aa, Artificial
  Synthetic peptide
KASQSLTHTDGTTALY

SEQ ID NO: 93 - protein, 7 aa, Artificial
  Synthetic peptide
EVSVRAS

SEQ ID NO: 94 - protein, 8 aa, Artificial
  Synthetic peptide
AQVAYYPT

SEQ ID NO: 95 - protein, 14 aa, Artificial
  Synthetic peptide
AGTSSDIGGYNSVS

SEQ ID NO: 96 - protein, 7 aa, Artificial
  Synthetic peptide
EVNKRAS

SEQ ID NO: 97 - protein, 10 aa, Artificial
  Synthetic peptide
ASYRSANNVV

SEQ ID NO: 98 - protein, 14 aa, Artificial
  Synthetic peptide
GLSSGSVTTNNYPG

SEQ ID NO: 99 - protein, 7 aa, Artificial
  Synthetic peptide
STSSRHS

SEQ ID NO: 100 - protein, 10 aa, Artificial
  Synthetic peptide
ALDIGSYTAV

SEQ ID NO: 101 - protein, 14 aa, Artificial
  Synthetic peptide
GLTSGSVTSSNYPG

SEQ ID NO: 102 - protein, 7 aa, Artificial
  Synthetic peptide
NTNSRHP

SEQ ID NO: 103 - protein, 10 aa, Artificial
  Synthetic peptide
ALHKGSYTAV

SEQ ID NO: 104 - protein, 14 aa, Artificial
  Synthetic peptide
VGSSSDVGYGDYVS

SEQ ID NO: 105 - protein, 7 aa, Artificial
  Synthetic peptide
DVEKRAS

SEQ ID NO: 106 - protein, 10 aa, Artificial
  Synthetic peptide
ASYRSDSNFV

SEQ ID NO: 107 - protein, 11 aa, Artificial
  Synthetic peptide
QASQSISSYLA

SEQ ID NO: 108 - protein, 7 aa, Artificial
  Synthetic peptide
GASRLEP

SEQ ID NO: 109 - protein, 9 aa, Artificial
  Synthetic peptide
LQDYSWPYS

SEQ ID NO: 110 - protein, 16 aa, Artificial
  Synthetic peptide
KASQSLIHIDGKTYLY

SEQ ID NO: 111 - protein, 7 aa, Artificial
  Synthetic peptide
QVSNHES

SEQ ID NO: 112 - protein, 8 aa, Artificial
  Synthetic peptide
AQATYYPS

SEQ ID NO: 113 - protein, 17 aa, Artificial
  Synthetic peptide
KSSQSVVSGSNQKSYLN

SEQ ID NO: 114 - protein, 7 aa, Artificial
  Synthetic peptide
YASTQES

SEQ ID NO: 115 - protein, 9 aa, Artificial
  Synthetic peptide
QQAYSAPYN

SEQ ID NO: 116 - protein, 16 aa, Artificial
  Synthetic peptide
KASQSLVHTDGKTYVY

SEQ ID NO: 117 - protein, 8 aa, Artificial
  Synthetic peptide
AQATYYPS

SEQ ID NO: 118 - protein, 13 aa, Artificial
  Synthetic peptide
TGSNRNIGNNYVN

SEQ ID NO: 119 - protein, 7 aa, Artificial
  Synthetic peptide
SDNLRTS

SEQ ID NO: 120 - protein, 11 aa, Artificial
  Synthetic peptide
SSWDDSLSGAV

SEQ ID NO: 121 - protein, 117 aa, Artificial
  Synthetic peptide
QVQLVESGGGLVQPGGSLRLSCAASGFIFINYGMHWVRQAPGKGLEWVSAVNSGGASTDYADSVKGRFTISRDDAKNTLYLQMNSLKSEDTAVYYCVKGWFYGIHYWGKGTLVTVSS

SEQ ID NO: 122 - protein, 111 aa, Artificial
  Synthetic peptide
QAVLTQLPSVSGSPGQKITISCTGSSSNIGGGYSVQWFQHLPGTPPKLLIYGNSNRASGVPDRFSGSKSGSSASLTITGLQAEDEADYYCESYDDWLKGRGFGGGSKLTVL

SEQ ID NO: 123 - protein, 124 aa, Artificial
  Synthetic peptide
QVQLVESGPGLVKPSQTLSLTCTVSGGSITTNYYSWIWIRQPPGKGLEWMGASVYSGSTFYSPSLKNTSISKDTAQNQFTLQLRSVTPEDTAVYYCARASSAHWGSSFISIDYWGQGTQVTVSS

SEQ ID NO: 124 - protein, 110 aa, Artificial
  Synthetic peptide
QSVLTQPPSVSGSPGKTVTISCAGTSSDVGYGNYVSWYQQLPGMAPKLLIYDVDIRASGIADRFSGSKSGNTASLTISGLQSEDEADYYCASYRTNNNAVFGGGTHLTVL

SEQ ID NO: 125 - protein, 5 aa, Artificial
  Synthetic peptide
NYGMH

SEQ ID NO: 126 - protein, 17 aa, Artificial
  Synthetic peptide
AVNSGGASTDYADSVKG

SEQ ID NO: 127 - protein, 8 aa, Artificial
  Synthetic peptide
GWFYGIHY

SEQ ID NO: 128 - protein, 7 aa, Artificial
  Synthetic peptide
TNYYSWI

SEQ ID NO: 129 - protein, 16 aa, Artificial
  Synthetic peptide
ASVYSGSTFYSPSLKN

SEQ ID NO: 130 - protein, 15 aa, Artificial
  Synthetic peptide
ASSAHWGSSFISIDY

SEQ ID NO: 131 - protein, 14 aa, Artificial
  Synthetic peptide
TGSSSNIGGGYSVQ

SEQ ID NO: 132 - protein, 7 aa, Artificial
  Synthetic peptide
GNSNRAS

SEQ ID NO: 133 - protein, 11 aa, Artificial
  Synthetic peptide
ESYDDWLKGRG

SEQ ID NO: 134 - protein, 14 aa, Artificial
  Synthetic peptide
AGTSSDVGYGNYVS

SEQ ID NO: 135 - protein, 7 aa, Artificial
  Synthetic peptide
DVDIRAS

SEQ ID NO: 136 - protein, 10 aa, Artificial
  Synthetic peptide
ASYRTNNNAV